European Patent Application EP 4 752 220 A1, published June 3, 2026. Title: COMBINATION FOR CRYSTALLINE NANOCELLULOSE PRODUCTION. Applicant: ASOCIACION CENTRO DE INVESTIGACION COOPERATIVA EN BIOCIENCIAS CIC bioGUNE. Application EP -. The sequence listing filed with the application follows.

SEQUENCE LISTING (36 sequences)

SEQ ID NO: 1 - protein, 297 aa, synthetic construct
  REGION 1..297: note = Endoglucanase catalytic domain
TPVETHGQLSVKGGQLVDENGKPVQLRGMSSHGLQWFGDFVNKDSMKWLRDDWGINVFRVAMYTAEGGYITNPSVKNKVKEAVEAAIDLGMYVIIDWHILSDNDPNTYKEQAKAFFQEMAAKYGNYPNVIYEICNEPNGGVTWSNQIKPYAEEVIPAIRANDPDNIIIVGTPTWSQDVHDAADNPLPYSNIMYALHFYAGTHGQSLRDKIDYALSKGVAIFVTEWGTSDASGNGGPFLNESQKWIDFMNSRNISWANWSLSDKSETSAALMPGASPTGGWTDSNLSASGKFVREQIR

SEQ ID NO: 2 - protein, 297 aa, synthetic construct
  REGION 1..297: note = Endoglucanase catalytic domain
TPVETHGQLSVKGGQLVDENGQPVQLRGMSSHGLQWYGDFVNKDSMKWLRDDWGINVFRVAMYTAEGGYITNPSVKNKVKEAVEAAIDLGLYVIIDWHILSDGDPNTYKEQAKAFFQEMATLYGNYPNVIYEICNEPNGNVTWSNQIKPYAEEVIPVIRANDPDNIIIVGTPTWSQDVHDAADNPLPYSNIMYALHFYAGTHGQSLRDKIDYALNKGAAIFVTEWGTSDASGNGGPFLNESQEWIDFMNSRNISWANWSLSDKSETSAALMPGASPTGGWTDSQLSASGKFVREQIR

SEQ ID NO: 3 - protein, 297 aa, synthetic construct
  REGION 1..297: note = Endoglucanase catalytic domain
TPVEINGQLQVCGVQLCNQYGKPIQLRGMSTHGIQWFGNCVNNASLDALANDWRADIFRIAMYIQEDGYETNPAGTNRVNNLVEEATARGMYVLIDWHILTPGDPNYNLDRAKTFFAEIAARHASKTNVIYEIANEPNGGVSWSNTIKSYAEEVIPVIRANDPDSVVIVGTRGWSSDSTEIVNNPVNASNIMYAFHFYAASHRDNYRDEVERAAARGLPVFVTEFGTVTYTGDGGNDLASSQKWLDLLDARKIGWANWNFSDKAESSAALRPGTCAGGSWTGTSLTPSGVFVRERIR

SEQ ID NO: 4 - protein, 297 aa, synthetic construct
  REGION 1..297: note = Endoglucanase catalytic domain
TPVETHGQLSVKGGQLVDENGKPVQLRGMSSHGLQWFGDFVNKDSMKWLRDDWGINVFRVAMYTAEDGYITNPSVKNKVKEAVEAAIDLGMYVIIDWHILSDNDPNTYKAQAKAFFQEMAALYGNYPNVIYEIANEPNGNVTWNNQIKPYAEEVIPVIRAKDPDNIIIVGTGTWSQDVHDAADNPLPDSNIMYALHFYAGTHGQFLRDRIDYALSKGAAIFVTEWGTSDASGNGGPFLPESQEWIDFMNSRKISWANWSLSDKSETSAALMPGASPTGGWTESQLSASGKFVREQIR

SEQ ID NO: 5 - protein, 122 aa, Phanerochaete carnosa
MTRFATVLFSLAVIGAASAAPAEKRSTTREGRGTWYDTGLGACGWNNVNSDTVIALSPSVYSGGSHCGQTVTVTNVVTGAKATGTVADECPGCGPNDIDMTPGLFQQLGSLDEGVLTVSWTL

SEQ ID NO: 6 - protein, 150 aa, synthetic construct
  REGION 1..150: note = Carbohydrate binding domain
QENGISVQYRAGDGSMNSNQIRPQLQIKNNGNTTVDLKDVTARYWYNAKNKGQNVDCDYAQLGCGNVTYKFVTLHKPKQGADTYLELGFKNGTLAPGASTGNIQLRLHNDDWSNYAQSGDYSFFKSNTFKTTKKITLYDQGKLIWGTEPN

SEQ ID NO: 7 - protein, 87 aa, synthetic construct
  REGION 1..87: note = Carbohydrate binding domain
FTVQWKKSSSWEEGGKKCGGYEIVITNNGDTVNSWTAKVTVPGNTKLMSQWNGIFSISGNTMTVKNESYNGTIEKGKSISFGFNYSA

SEQ ID NO: 8 - protein, 87 aa, synthetic construct
  REGION 1..87: note = Carbohydrate binding domain
YQLKVTVSSSWESGDGYGGTYSLSFTNRSAAVKAWDAQIEVPEGSKVTEAWGCETGIDGTILTVTAKDWGAAVAKGSTVEIGFNMDT

SEQ ID NO: 9 - protein, 84 aa, synthetic construct
  REGION 1..84: note = Carbohydrate binding domain
YKADFKVVNSWEEGGKKCYQLSGTLTNLSSSISSWTVVFDAGNGAEIKQFWNSKCTISGNKITVGPADYNSRIGTGASVSDVGM

SEQ ID NO: 10 - protein, 87 aa, synthetic construct
  REGION 1..87: note = Carbohydrate binding domain
FYAEIGHDSTWEASGKTCATENINIYNKTSSVSGWKLDVIYKGKPAIEDIWNGEKKINEYTVSITPADYNQDIPAGGSVNVGYNIAS

SEQ ID NO: 11 - protein, 87 aa, synthetic construct
  REGION 1..87: note = Carbohydrate binding domain
YYASISDNSSWQENGKNAATKNVIIYNKDKKVTGWKIELVFASEPELADIWGGKAEVNGDTITVVGYDYTAELKAGGNVNFGFNVKA

SEQ ID NO: 12 - protein, 77 aa, synthetic construct
  REGION 1..77: note = Carbohydrate binding domain
WAEQNQTAFQYELLFSNQSEAFGTWKVILDTGKEVKVQNSWNCSLEADGNLLTFTPADYNAKLAKGAEMADVGMILV

SEQ ID NO: 13 - protein, 85 aa, synthetic construct
  REGION 1..85: note = Carbohydrate binding domain
MQFKQSNSWEGNGRFYAQYDLIIDNKEDVISDWTFKINTTNGTTLEQSWNCTVDTSDLQWSVVPVDYNKIIESQAQMNNVGFIIS

SEQ ID NO: 14 - protein, 147 aa, synthetic construct
  REGION 1..147: note = Carbohydrate binding domain
NGISVQYRAGDGSMNSNQIRPQLQIKNNGNTTVDLKDVTARYWYNAKNKGQNVDCDYAQLGCGNVTYKFVTLHKPKQGADTYLELGFKNGTLAPGASTGNIQLRLHNDDWSNYAQSGDYSFFKSNTFKTTKKITLYDQGKLIWGTEP

SEQ ID NO: 15 - protein, 137 aa, synthetic construct
  REGION 1..137: note = Carbohydrate binding domain
NGISVQYRAGDGSMNSNQIRPQLQIKNNGNTTVDLKDVTARYWYKAKNKGQNVDCDYAQIGCGNVTYKFVTLHKPKQGADTYLELGFKNGTLAPGASTGNIQLRLHNDDWSNYAQSGDYSFFKSNTFKTTKKITLYD

SEQ ID NO: 16 - protein, 147 aa, synthetic construct
  REGION 1..147: note = Carbohydrate binding domain
NGISVQYKAGDGGVNSNQIRPQLHIKNNGNATVDLKDVTARYWYNAKNKGQNFDCDYAQIGCGNLTHKFVTLHKPKQGADTYLELGFKTGTLSPGASTGNIQLRLHNDDWSNYAQSDDYSFFQSNTFKTTKKITLYHQGKLIWGTEP

SEQ ID NO: 17 - protein, 63 aa, synthetic construct
  REGION 1..63: note = Carbohydrate binding domain
PGEPEPDPGEPDPTPPSDGDYPAWDPNTIYTDEIVYHNGQLWQAKWWTQNQEPGDYGPWEPLN

SEQ ID NO: 18 - protein, 145 aa, synthetic construct
  REGION 1..145: note = Carbohydrate binding domain
GNLVVQYKVGDTSATDNQMKPSFNIKNNGTTPVNLSGLKLRYYFTKDGTDMSASIDWAQIGASNISAAFADFTGSNTDTYVELSFSAGSIPAGGQTGDIQLRMYKTDWSNFNEANDYSYDGAKTYADWNRVTLHQNGTLVWGTTP

SEQ ID NO: 19 - protein, 57 aa, synthetic construct
  REGION 1..57: note = Carbohydrate binding domain
DPGEPDPTPPSDGEYPAWDPNQIYTNEIVYHNGQLWQAKWWTQNQEPGDYGPWEPLN

SEQ ID NO: 20 - protein, 144 aa, synthetic construct
  REGION 1..144: note = Carbohydrate binding domain
GSLVLQYRAADTNAGDNAIKPHFNIRNTGASPVDLSGVKLRYYFTKDGIPLSFAVDWAQVGSPNVKGTFGSASGAGADTYLEVSFTGSIPAGGQTGEIQTRIHKSDWSSFQESGDYSYDPGKTYADWSKVTLYRDGTRVWGVEP

SEQ ID NO: 21 - protein, 147 aa, synthetic construct
  REGION 1..147: note = Carbohydrate binding domain
NITSAVYTISNTDPVKQVSAPTFSLQSAQTVTLTSSDNDSVIHYTTDGTPTSSSPVYTNMTDSSVVTNTYTITNETSNSPVEVEVEYKTTVKVTLTNNSSTPINGWKLSWINNMWTANYSIKDSAIVKDYNNIIPANGGTQIFGFSI

SEQ ID NO: 22 - protein, 147 aa, synthetic construct
  REGION 1..147: note = Carbohydrate binding domain
QGIVLQYRTGDTNTKDNAIRPEFNIKNTGNTAVKLSDLKIRYYYTDESKGQQLFVDWAKVGNEKVKATFVALPEPKAKADKYVEISFTDGTIQPGGESGEIQPRIHAANWSNFDETNDYSYGASQTFANWDHATVYQQGKLVWGIEP

SEQ ID NO: 23 - protein, 147 aa, synthetic construct
  REGION 1..147: note = Carbohydrate binding domain
EGIVLQYRTDDTNAKDNAIRPQFNIKNTGKTAVKLSDLKIRYYYTDESKAQQFFVDWAKIGNEKVKATFVTLPNPKSKADKYVEISFTDGTIQPGGETGEIQSRIHAANWSNFDETNDYSYGAAQTFADWDHGTVYQQGKLVWGIEP

SEQ ID NO: 24 - protein, 107 aa, synthetic construct
  REGION 1..107: note = Carbohydrate binding domain
QAAGLTATVTKESSWDNGYSASVTVRNDTSSVSQWEVVLTLPGGTTVAQVWNAQHTSSGNSHTFTGVSWNSTIPPGGTASFGFIASGSGEPTHCTINGAPCDEGSEP

SEQ ID NO: 25 - protein, 106 aa, synthetic construct
  REGION 1..106: note = Carbohydrate binding domain
AATGCSVTYTTNSWSNGFTANVTVTNLGDAIGNWTLGFSFPSGQRVTQGWSAIWSQSGNAVTARSESWNGNLATGASTSIGFNGSFTGSPTSFTLNGVPCTGSTTT

SEQ ID NO: 26 - protein, 103 aa, synthetic construct
  REGION 1..103: note = Carbohydrate binding domain
EAASFTVTNSWSTGYQGEVTVSNPASSINTWKVQLTLPAGSTIGQAWNATLATGGQTFTFTPAGWNGTIAGGSATSFGFVVTGTGRPTSCTVNGQACTGLTGA

SEQ ID NO: 27 - protein, 107 aa, synthetic construct
  REGION 1..107: note = Carbohydrate binding domain
AATGCHVDYTVTNQWQGGFQAAVKVTNLGDAITGWLLRFTFPAGQKVAQGWNATWAQSGATATAANADWNRTLTTGATTELGFTGTTTGVPASFTLNGVTCTGSTTT

SEQ ID NO: 28 - protein, 106 aa, synthetic construct
  REGION 1..106: note = Carbohydrate binding domain
AATGCAVTYTTNSWQGGFTATVAVRNLGDPVSNWTLGFTFPGGQRVVQGWSATWQQSGSAVTARSLDYNGALGTGASTTIGFNGSWTGSPTSFTLNGTVCTGGTST

SEQ ID NO: 29 - protein, 106 aa, synthetic construct; identical to SEQ ID NO: 28
  REGION 1..106: note = Carbohydrate binding domain

SEQ ID NO: 30 - protein, 100 aa, synthetic construct
  REGION 1..100: note = Carbohydrate binding domain
ESENATISRGVVEANHTGFTGSGFVNYDNVTGSYVEYTVNAAQAGPHTLTFRYANGTTANRPLDITVNGSIAVDDLGFAGTGAWSTVTTTVNLAAGSNKI

SEQ ID NO: 31 - protein, 107 aa, synthetic construct
  REGION 1..107: note = Carbohydrate binding domain
NAAGCRVDYTVTNQWQGGFQAGVKITNLGDTVRGWTLKFTLPTGQKVVQGWSAAWSQSGSTVTVAGADWNGTLATGASADTGFVGSFTGKPTAFTLNGVACTGSVDD

SEQ ID NO: 32 - protein, 105 aa, synthetic construct
  REGION 1..105: note = Carbohydrate binding domain
AATGCKAEYTITSQWEGGFQAGVKITNLGDPVSGWTLGFTMPAGQRLVQGWNATWSQSGSAVTAGGVDWNRTLATGASADLGFVGSFTGAPTSFTLNGATCSGSV

SEQ ID NO: 33 - protein, 81 aa, synthetic construct
  REGION 1..81: note = Carbohydrate binding domain
DGIQTESTTDTGGGLNIGWTDAGDWTSPAAGRYKVSYRNSGMLQLEAAGGFPTYGSITGGWQSWQTISHEVNLNWIKVEPA

SEQ ID NO: 34 - protein, 81 aa, synthetic construct
  REGION 1..81: note = Carbohydrate binding domain
PTEPTNPGNGTTGDVVLQYRNVDNNPSDDAIRMAVNIKNTGSTPIKLSDLQVRYYFHDDGKPGANLFVDWANVGPNNIVTS

SEQ ID NO: 35 - protein, 81 aa, synthetic construct
  REGION 1..81: note = Carbohydrate binding domain
PTEPTNPGNGTTGDIVLQYRNVDNNPSDDAIRMAFNIKNTGSTPIKLSDLQVRYYFHDDGKPGANLFVDWANVGPNNIVTS

SEQ ID NO: 36 - protein, 15 aa, synthetic construct
  REGION 1..15: note = Linking domain
GTKDIPETPAKDKPT